European Patent Specification EP 3 406 634 B1, published June 5, 2024. Title: ANTIBODIES COMPRISING CHIMERIC CONSTANT DOMAINS. Applicant: Regeneron Pharmaceuticals, Inc. Application EP14706169.1. The sequence listing filed with the application follows.

SEQUENCE LISTING (44 sequences)

SEQ ID NO: 1 - protein, 232 aa, Artificial sequence
  Synthetic
DKRVESKYGPPCPPCPAPPVAGPSVFLFPPKPKDTLMISRTPEVTCVVVDVSQEDPEVQFNWYVDGVEVHNAKTKPREEQFNSTYRVVSVLTVLHQDWLNGKEYKCKVSNKGLPSSIEKTISKAKGQPREPQVYTLPPSQEEMTKNQVSLTCLVKGFYPSDIAVEWESNGQPENNYKTTPPVLDSDGSFFLYSRLTVDKSRWQEGNVFSCSVMHEALHNHYTQKSLSLSLGK

SEQ ID NO: 2 - protein, 235 aa, Artificial sequence
  Synthetic
DKKVEPKSCDKTHTCPPCPAPPVAGPSVFLFPPKPKDTLMISRTPEVTCVVVDVSQEDPEVQFNWYVDGVEVHNAKTKPREEQFNSTYRVVSVLTVLHQDWLNGKEYKCKVSNKGLPSSIEKTISKAKGQPREPQVYTLPPSRDELTKNQVSLTCLVKGFYPSDIAVEWESNGQPENNYKTTPPVLDSDGSFFLYSKLTVDKSRWQQGNVFSCSVMHEALHNHYTQKSLSLSPGK

SEQ ID NO: 3 - protein, 8 aa, Homo sapiens
PCPAPPVA

SEQ ID NO: 4 - protein, 4 aa, Homo sapiens
DKKV

SEQ ID NO: 5 - protein, 4 aa, Homo sapiens
DKRV

SEQ ID NO: 6 - protein, 12 aa, Homo sapiens
EPKSCDKTHTCP

SEQ ID NO: 7 - protein, 9 aa, Homo sapiens
ESKYGPPCP

SEQ ID NO: 8 - protein, 20 aa, Artificial sequence
  Synthetic
EPKSCDKTHTCPPCPAPPVA

SEQ ID NO: 9 - protein, 17 aa, Artificial sequence
  Artificial sequence
ESKYGPPCPPCPAPPVA

SEQ ID NO: 10 - protein, 104 aa, Homo sapiens
GPSVFLFPPKPKDTLMISRTPEVTCVVVDVSQEDPEVQFNWYVDGVEVHNAKTKPREEQFNSTYRVVSVLTVLHQDWLNGKEYKCKVSNKGLPSSIEKTISKAK

SEQ ID NO: 11 - protein, 107 aa, Homo sapiens
GQPREPQVYTLPPSRDELTKNQVSLTCLVKGFYPSDIAVEWESNGQPENNYKTTPPVLDSDGSFFLYSKLTVDKSRWQQGNVFSCSVMHEALHNHYTQKSLSLSPGK

SEQ ID NO: 12 - protein, 107 aa, Homo sapiens
GQPREPQVYTLPPSQEEMTKNQVSLTCLVKGFYPSDIAVEWESNGQPENNYKTTPPVLDSDGSFFLYSRLTVDKSRWQEGNVFSCSVMHEALHNHYTQKSLSLSLGK

SEQ ID NO: 13 - protein, 330 aa, Homo sapiens [sequence omitted]

SEQ ID NO: 14 - protein, 326 aa, Homo sapiens
ASTKGPSVFPLAPCSRSTSESTAALGCLVKDYFPEPVTVSWNSGALTSGVHTFPAVLQSSGLYSLSSVVTVPSSNFGTQTYTCNVDHKPSNTKVDKTVERKCCVECPPCPAPPVAGPSVFLFPPKPKDTLMISRTPEVTCVVVDVSHEDPEVQFNWYVDGVEVHNAKTKPREEQFNSTFRVVSVLTVVHQDWLNGKEYKCKVSNKGLPAPIEKTISKTKGQPREPQVYTLPPSREEMTKNQVSLTCLVKGFYPSDISVEWESNGQPENNYKTTPPMLDSDGSFFLYSKLTVDKSRWQQGNVFSCSVMHEALHNHYTQKSLSLSPGK

SEQ ID NO: 15 - protein, 327 aa, Homo sapiens
ASTKGPSVFPLAPCSRSTSESTAALGCLVKDYFPEPVTVSWNSGALTSGVHTFPAVLQSSGLYSLSSVVTVPSSSLGTKTYTCNVDHKPSNTKVDKRVESKYGPPCPSCPAPEFLGGPSVFLFPPKPKDTLMISRTPEVTCVVVDVSQEDPEVQFNWYVDGVEVHNAKTKPREEQFNSTYRVVSVLTVLHQDWLNGKEYKCKVSNKGLPSSIEKTISKAKGQPREPQVYTLPPSQEEMTKNQVSLTCLVKGFYPSDIAVEWESNGQPENNYKTTPPVLDSDGSFFLYSRLTVDKSRWQEGNVFSCSVMHEALHNHYTQKSLSLSLGK

SEQ ID NO: 16 - DNA, 60 bp, Artificial sequence
  Synthetic
ttcgcgcagcttaggtttatgccaggggggacgggtggcacgggtcgtggtggacaccgt

SEQ ID NO: 17 - DNA, 40 bp, Artificial sequence
  Synthetic
aagcttatactcgagctctagattgggaacccgggtctct

SEQ ID NO: 18 - DNA, 58 bp, Artificial sequence
  Synthetic
cccaccgtgcccagcaccacctgtggcaggaccatcagtcttcctgttccccccaaaa

SEQ ID NO: 19 - DNA, 44 bp, Artificial sequence
  Synthetic
tgtgtcttcagggagagggacagagacccatttactcgccggcg

SEQ ID NO: 20 - DNA, 60 bp, Artificial sequence
  Synthetic
ctcgggtttagaacactgttttgagtgtgtacgggtggcacgggtcgtggtggacaccgt

SEQ ID NO: 21 - DNA, 51 bp, Artificial sequence
  Synthetic
aaatcttgtgacaaaactcacacatgcccaccgtgcccagcaccacctgtg

SEQ ID NO: 22 - DNA, 54 bp, Artificial sequence
  Synthetic
gagaaaaccatctccaaagccaaagggcagccccgagaaccacaggtgtacacc

SEQ ID NO: 23 - DNA, 54 bp, Artificial sequence
  Synthetic
ctcttttggtagaggtttcggtttcccgtcggggctcttggtgtccacatgtgg

SEQ ID NO: 24 - DNA, 39 bp, Artificial sequence
  Artificial
cttcagggagagggacagaggcccatttactcgccggcg

SEQ ID NO: 25 - DNA, 20 bp, Artificial sequence
  Synthetic
gctgacagactaacagactg

SEQ ID NO: 26 - DNA, 24 bp, Artificial sequence
  Synthetic
gacctcaggggtccgggagatcat

SEQ ID NO: 27 - DNA, 26 bp, Artificial sequence
  Synthetic
atacattatacgaagttataccggta

SEQ ID NO: 28 - DNA, 990 bp, Artificial sequence
  Synthetic
gcctccaccaagggcccatcggtcttccccctggcaccctcctccaagagcacctctgggggcacagcggccctgggctgcctggtcaaggactacttccccgaaccggtgacggtgtcgtggaactcaggcgccctgaccagcggcgtgcacaccttcccggctgtcctacagtcctcaggactctactccctcagcagcgtggtgaccgtgccctccagcagcttgggcacccagacctacatctgcaacgtgaatcacaagcccagcaacaccaaggtggacaagaaagttgagcccaaatcttgtgacaaaactcacacatgcccaccgtgcccagcaccacctgtggcaggaccatcagtcttcctgttccccccaaaacccaaggacactctcatgatctcccggacccctgaggtcacgtgcgtggtggtggacgtgagccaggaagaccccgaggtccagttcaactggtacgtggatggcgtggaggtgcataatgccaagacaaagccgcgggaggagcagttcaacagcacgtaccgtgtggtcagcgtcctcaccgtcctgcaccaggactggctgaacggcaaggagtacaagtgcaaggtctccaacaaaggcctcccgtcctccatcgagaaaaccatctccaaagccaaagggcagccccgagaaccacaggtgtacaccctgcccccatcccgggatgagctgaccaagaaccaggtcagcctgacctgcctggtcaaaggcttctatcccagcgacatcgccgtggagtgggagagcaatgggcagccggagaacaactacaagaccacgcctcccgtgctggactccgacggctccttcttcctctacagcaagctcaccgtggacaagagcaggtggcagcaggggaacgtcttctcatgctccgtgatgcatgaggctctgcacaaccactacacgcagaagtccctctccctgtctccgggtaaatga

SEQ ID NO: 29 - DNA, 981 bp, Artificial sequence
  Synthetic
gccagcacaaaaggtcctagcgtttttccacttgccccatgttcaaggtcaacctccgaaagtaccgccgctcttggctgtctcgtaaaagattattttcccgaacctgtaactgtctcctggaactccggcgcactcacttccggcgtacataccttccccgctgtcctccaatcttccggtctctactccctgtcttctgttgtcactgttccatcatcctcactcggcacaaaaacatatacctgcaacgttgatcacaagccaagtaataccaaagttgataagcgcgtcgaatccaaatacggtcccccctgcccaccgtgcccagcaccacctgtggcaggaccatcagtcttcctgttccccccaaaacccaaggacactctcatgatctcccggacccctgaggtcacgtgcgtggtggtggacgtgagccaggaagaccccgaggtccagttcaactggtacgtggatggcgtggaggtgcataatgccaagacaaagccgcgggaggagcagttcaacagcacgtaccgtgtggtcagcgtcctcaccgtcctgcaccaggactggctgaacggcaaggagtacaagtgcaaggtctccaacaaaggcctcccgtcctccatcgagaaaaccatctccaaagccaaagggcagccccgagagccacaggtgtacaccctgcccccatcccaggaggagatgaccaagaaccaggtcagcctgacctgcctggtcaaaggcttctaccccagcgacatcgccgtggagtgggagagcaatgggcagccggagaacaactacaagaccacgcctcccgtgctggactccgacggctccttcttcctctacagcaggctcaccgtggacaagagcaggtggcaggaggggaatgtcttctcatgctccgtgatgcatgaggctctgcacaaccactacacacagaagtccctctccctgtctctgggtaaatga

SEQ ID NO: 30 - protein, 329 aa, Artificial sequence
  Synthetic
ASTKGPSVFPLAPSSKSTSGGTAALGCLVKDYFPEPVTVSWNSGALTSGVHTFPAVLQSSGLYSLSSVVTVPSSSLGTQTYICNVNHKPSNTKVDKKVEPKSCDKTHTCPPCPAPPVAGPSVFLFPPKPKDTLMISRTPEVTCVVVDVSQEDPEVQFNWYVDGVEVHNAKTKPREEQFNSTYRVVSVLTVLHQDWLNGKEYKCKVSNKGLPSSIEKTISKAKGQPREPQVYTLPPSRDELTKNQVSLTCLVKGFYPSDIAVEWESNGQPENNYKTTPPVLDSDGSFFLYSKLTVDKSRWQQGNVFSCSVMHEALHNHYTQKSLSLSPGK

SEQ ID NO: 31 - protein, 326 aa, Artificial sequence
  Synthetic
ASTKGPSVFPLAPCSRSTSESTAALGCLVKDYFPEPVTVSWNSGALTSGVHTFPAVLQSSGLYSLSSVVTVPSSSLGTKTYTCNVDHKPSNTKVDKRVESKYGPPCPPCPAPPVAGPSVFLFPPKPKDTLMISRTPEVTCVVVDVSQEDPEVQFNWYVDGVEVHNAKTKPREEQFNSTYRVVSVLTVLHQDWLNGKEYKCKVSNKGLPSSIEKTISKAKGQPREPQVYTLPPSQEEMTKNQVSLTCLVKGFYPSDIAVEWESNGQPENNYKTTPPVLDSDGSFFLYSRLTVDKSRWQEGNVFSCSVMHEALHNHYTQKSLSLSLGK

SEQ ID NO: 32 - DNA, 708 bp, Artificial sequence
  Synthetic
gacaagaaagttgagcccaaatcttgtgacaaaactcacacatgcccaccgtgcccagcaccacctgtggcaggaccatcagtcttcctgttccccccaaaacccaaggacactctcatgatctcccggacccctgaggtcacgtgcgtggtggtggacgtgagccaggaagaccccgaggtccagttcaactggtacgtggatggcgtggaggtgcataatgccaagacaaagccgcgggaggagcagttcaacagcacgtaccgtgtggtcagcgtcctcaccgtcctgcaccaggactggctgaacggcaaggagtacaagtgcaaggtctccaacaaaggcctcccgtcctccatcgagaaaaccatctccaaagccaaagggcagccccgagaaccacaggtgtacaccctgcccccatcccgggatgagctgaccaagaaccaggtcagcctgacctgcctggtcaaaggcttctatcccagcgacatcgccgtggagtgggagagcaatgggcagccggagaacaactacaagaccacgcctcccgtgctggactccgacggctccttcttcctctacagcaagctcaccgtggacaagagcaggtggcagcaggggaacgtcttctcatgctccgtgatgcatgaggctctgcacaaccactacacgcagaagtccctctccctgtctccgggtaaatga

SEQ ID NO: 33 - DNA, 699 bp, Artificial sequence
  Synthetic
gataagcgcgtcgaatccaaatacggtcccccctgcccaccgtgcccagcaccacctgtggcaggaccatcagtcttcctgttccccccaaaacccaaggacactctcatgatctcccggacccctgaggtcacgtgcgtggtggtggacgtgagccaggaagaccccgaggtccagttcaactggtacgtggatggcgtggaggtgcataatgccaagacaaagccgcgggaggagcagttcaacagcacgtaccgtgtggtcagcgtcctcaccgtcctgcaccaggactggctgaacggcaaggagtacaagtgcaaggtctccaacaaaggcctcccgtcctccatcgagaaaaccatctccaaagccaaagggcagccccgagagccacaggtgtacaccctgcccccatcccaggaggagatgaccaagaaccaggtcagcctgacctgcctggtcaaaggcttctaccccagcgacatcgccgtggagtgggagagcaatgggcagccggagaacaactacaagaccacgcctcccgtgctggactccgacggctccttcttcctctacagcaggctcaccgtggacaagagcaggtggcaggaggggaatgtcttctcatgctccgtgatgcatgaggctctgcacaaccactacacacagaagtccctctccctgtctctgggtaaatga

SEQ ID NO: 34 - DNA, 357 bp, Artificial sequence
  Synthetic
gacgtccaactggtgcagtcaggggctgaagtgaaaaaacctggggcctcagtgaaggtgtcctgcaaggcttctggctacacctttactaggtacacgatgcactgggtaaggcaggcacctggacagggtctggaatggattggatacattaatcctagccgtggttatactaattacgcagacagcgtcaagggccgcttcacaatcactacagacaaatccaccagcacagcctacatggaactgagcagcctgcgttctgaggacactgcaacctattactgtgcaagatattatgatgatcattactgccttgactactggggccaaggcaccacggtcaccgtctcctca

SEQ ID NO: 35 - DNA, 990 bp, Artificial sequence
  Synthetic
gcctccaccaagggcccatcggtcttccccctggcaccctcctccaagagcacctctgggggcacagcggccctgggctgcctggtcaaggactacttccccgaaccggtgacggtgtcgtggaactcaggcgccctgaccagcggcgtgcacaccttcccggctgtcctacagtcctcaggactctactccctcagcagcgtggtgaccgtgccctccagcagcttgggcacccagacctacatctgcaacgtgaatcacaagcccagcaacaccaaggtggacaagaaagttgagcccaaatcttgtgacaaaactcacacatgcccaccgtgcccagcaccacctgtggcaggaccatcagtcttcctgttccccccaaaacccaaggacactctcatgatctcccggacccctgaggtcacgtgcgtggtggtggacgtgagccaggaagaccccgaggtccagttcaactggtacgtggatggcgtggaggtgcataatgccaagacaaagccgcgggaggagcagttcaacagcacgtaccgtgtggtcagcgtcctcaccgtcctgcaccaggactggctgaacggcaaggagtacaagtgcaaggtctccaacaaaggcctcccgtcctccatcgagaaaaccatctccaaagccaaagggcagccccgagaaccacaggtgtacaccctgcccccatcccgggatgagctgaccaagaaccaggtcagcctgacctgcctggtcaaaggcttctatcccagcgacatcgccgtggagtgggagagcaatgggcagccggagaacaactacaagaccacgcctcccgtgctggactccgacggctccttcttcctctacagcaagctcaccgtggacaagagcaggtggcagcaggggaacgtcttctcatgctccgtgatgcatgaggctctgcacaacagattcacgcagaagtccctctccctgtctccgggtaaatga

SEQ ID NO: 36 - DNA, 981 bp, Artificial sequence
  Synthetic
gccagcacaaaaggtcctagcgtttttccacttgccccatgttcaaggtcaacctccgaaagtaccgccgctcttggctgtctcgtaaaagattattttcccgaacctgtaactgtctcctggaactccggcgcactcacttccggcgtacataccttccccgctgtcctccaatcttccggtctctactccctgtcttctgttgtcactgttccatcatcctcactcggcacaaaaacatatacctgcaacgttgatcacaagccaagtaataccaaagttgataagcgcgtcgaatccaaatacggtcccccctgcccaccgtgcccagcaccacctgtggcaggaccatcagtcttcctgttccccccaaaacccaaggacactctcatgatctcccggacccctgaggtcacgtgcgtggtggtggacgtgagccaggaagaccccgaggtccagttcaactggtacgtggatggcgtggaggtgcataatgccaagacaaagccgcgggaggagcagttcaacagcacgtaccgtgtggtcagcgtcctcaccgtcctgcaccaggactggctgaacggcaaggagtacaagtgcaaggtctccaacaaaggcctcccgtcctccatcgagaaaaccatctccaaagccaaagggcagccccgagagccacaggtgtacaccctgcccccatcccaggaggagatgaccaagaaccaggtcagcctgacctgcctggtcaaaggcttctaccccagcgacatcgccgtggagtgggagagcaatgggcagccggagaacaactacaagaccacgcctcccgtgctggactccgacggctccttcttcctctacagcaggctcaccgtggacaagagcaggtggcaggaggggaatgtcttctcatgctccgtgatgcatgaggctctgcacaacagattcacacagaagtccctctccctgtctctgggtaaatga

SEQ ID NO: 37 - protein, 329 aa, Artificial sequence
  Synthetic
ASTKGPSVFPLAPSSKSTSGGTAALGCLVKDYFPEPVTVSWNSGALTSGVHTFPAVLQSSGLYSLSSVVTVPSSSLGTQTYICNVNHKPSNTKVDKKVEPKSCDKTHTCPPCPAPPVAGPSVFLFPPKPKDTLMISRTPEVTCVVVDVSQEDPEVQFNWYVDGVEVHNAKTKPREEQFNSTYRVVSVLTVLHQDWLNGKEYKCKVSNKGLPSSIEKTISKAKGQPREPQVYTLPPSRDELTKNQVSLTCLVKGFYPSDIAVEWESNGQPENNYKTTPPVLDSDGSFFLYSKLTVDKSRWQQGNVFSCSVMHEALHNRFTQKSLSLSPGK

SEQ ID NO: 38 - protein, 326 aa, Artificial sequence
  Synthetic
ASTKGPSVFPLAPCSRSTSESTAALGCLVKDYFPEPVTVSWNSGALTSGVHTFPAVLQSSGLYSLSSVVTVPSSSLGTKTYTCNVDHKPSNTKVDKRVESKYGPPCPPCPAPPVAGPSVFLFPPKPKDTLMISRTPEVTCVVVDVSQEDPEVQFNWYVDGVEVHNAKTKPREEQFNSTYRVVSVLTVLHQDWLNGKEYKCKVSNKGLPSSIEKTISKAKGQPREPQVYTLPPSQEEMTKNQVSLTCLVKGFYPSDIAVEWESNGQPENNYKTTPPVLDSDGSFFLYSRLTVDKSRWQEGNVFSCSVMHEALHNRFTQKSLSLSLGK

SEQ ID NO: 39 - DNA, 41 bp, Artificial sequence
  Synthetic
gtgagcgctcttcggcagacgtccaactggtgcagtcaggg

SEQ ID NO: 40 - DNA, 47 bp, Artificial sequence
  Synthetic
cagctagctcttccggctgaggagacggtgaccgtggtgccttggcc

SEQ ID NO: 41 - protein, 107 aa, Artificial sequence
  Synthetic
GQPREPQVYTLPPSRDELTKNQVSLTCLVKGFYPSDIAVEWESNGQPENNYKTTPPVLDSDGSFFLYSKLTVDKSRWQQGNVFSCSVMHEALHNRFTQKSLSLSPGK

SEQ ID NO: 42 - protein, 107 aa, Artificial sequence
  Synthetic
GQPREPQVYTLPPSQEEMTKNQVSLTCLVKGFYPSDIAVEWESNGQPENNYKTTPPVLDSDGSFFLYSRLTVDKSRWQEGNVFSCSVMHEALHNRFTQKSLSLSLGK

SEQ ID NO: 43 - protein, 98 aa, Homo sapiens
ASTKGPSVFPLAPSSKSTSGGTAALGCLVKDYFPEPVTVSWNSGALTSGVHTFPAVLQSSGLYSLSSVVTVPSSSLGTQTYICNVNHKPSNTKVDKKV

SEQ ID NO: 44 - protein, 98 aa, Homo sapiens
ASTKGPSVFPLAPCSRSTSESTAALGCLVKDYFPEPVTVSWNSGALTSGVHTFPAVLQSSGLYSLSSVVTVPSSSLGTKTYTCNVDHKPSNTKVDKRV